European Patent Specification EP 3 865 581 B1, published September 25, 2024. Title: HUMANIZED UNIVERSAL LIGHT CHAIN MICE. Applicant: Regeneron Pharmaceuticals, Inc. Application To be assigned. The sequence listing filed with the application follows.

SEQUENCE LISTING (91 sequences)

SEQ ID NO: 1 - protein, 754 aa, Mus musculus
MLSLTWGMRLVERPVVPRVLLLLFALWLLLLVPVWCSQGHPTWRYISSEVVIPRKEIYHTKGLQAQRLLSYSLRFRGQRHIIHLRRKTLIWPRHLLLTTQDDQGALQMEYPFFPVDCYYIGYLEGILQSMVTVDTCYGGLSGVIKLDNLTYEIKPLNDSQSFEHLVSQIVSESDDTGPMNAWKHWSHNTGSPSSRLEYADGAPRLSSKNYATHPAAIKGHFQATHSVYSASGGDKLSSTVEYLFKVISLMDTYLTNLHMRYYVFLMTVYTEADPFSQDFRVPGGQAHTFYERVFYAHFRPDAGAIINKNSPGDDAVNPAERSICSPSALICLGQHGRNPLFLSIIITNRVGRSLGLKHDEGYCICQRRNTCIMFKNPQLTDAFSNCSLAEISNILNTPDLMPCLFYDRHVYYNTSLTYKFCGNFKVDNNEQCDCGSQKACYSDPCCGNDCRLTPGSICDKELCCANCTYSPSGTLCRPIQNICDLPEYCSGSKFICPDDTYLQDGTPCSEEGYCYKGNCTDRNIQCMEIFGVSAKNANIKCYDINKQRFRFGHCTRAEESLTFNACADQDKLCGRLQCTNVTNLPFLQEHVSFHQSVISGVTCFGLDEHRGTETADAGLVRHGTPCSRGKFCDRGACNGSLSRLGYDCTPEKCNFRGVCNNRRNCHCHFGWSPPKCKEEGHSGSIDSGSPPVQRRIIKQNLEPVVYLRILFGRIYFLFVALLFGIATRVGVTKIFRFEDLQAALRSWQEQAKDK

SEQ ID NO: 2 - protein, 756 aa, Mus musculus
MLSLTWGMRLVERPVVPRVLLLLFALWLLLLVPVWCSQGHPTWRYISSEVVIPRKEIYHTKGLQAQRLLSYSLHFRGQRHIIHLRRKTLIWPRHLLLTTQDDQGALQMDYPFFPVDCYYIGYLEGIPQSMVTVDTCYGGLSGVMKLDDLTYEIKPLNDSQSFEHLVSQIVSESDDTGPMNAWKHWSHNTGSPSSRLEYADGAPRISSKNYATHPAAIKGHFQATNSVYNSAAGDKLSSTVGYLFQVISLMDTYLTNLHMRYYVFLMTVYTNSDPFRLEFAVPGGSAYNYYVSVFYNKFKPDAGVLLNKYGPQDNQVNPAERSICSSLALICIGKYDRNPLFLSPIITNRVGRSLGLKYDEGYCVCQRRNTCIMFRHPQLTDAFSNCSLAEISNILNTPGLMPCLFYDRHVYYNTSLTYKFCGNFKVDNDEQCDCGSQKACYSDPCCGNDCRLTPGSICDKELCCANCTYSPSGTLCRPIQNICDLPEYCNGTKYICPDDTYLQDGTPCSEDGYCYKGNCTDRNIQCMEIFGVSAKNANIKCYDINKQRFRFGHCTRAEESLTFNACADQDKLCGRLQCTNVTNLPYLQEHVSFHQSIISGFTCFGLDEHRGTETTDAGMVRHGTPCSKSKFCDQGACSGSLSHLGYDCTPEKCSFRGVCNNHRNCHCHFGWKPPECKEEGLSGSIDSGSPPVQRHTIKQKQEPVVYLRILFGRIYFLFVALLFGIATRVGVTKIFRFEDLQATLRSGQGPARDKPK

SEQ ID NO: 3 - DNA, 13894 bp, Artificial Sequence
  synthetic
gtcctaaggtagcgagggatgacagattctctgttcagtgcactcagggtctgcctccacgagaatcaccatgccctttctcaagactgtgttctgtgcagtgccctgtcagtggaaatctggagagcatgcttccatgagcttgtgagtagtatatctagtaagccatggctttgtgttaatggtgatgttctacataccagttctctggcttaataatgaggtgatgattctatgttcctgtaacgcttcctcaactgggtcctaagtctttcttcactccatctattcctctaaggaatgatcctgaaaatcccatcacaaactataggagatgggaaccatcaaaaaacacagtgacaaagaggtgggaacgcatcagggttcaggaaccatattttaaaaagatatcgtaaataacttcttaaaagagatatagacaaatctccattaatacggagaccagaggcctaaggctaagaaccaatggtggctcaaggtctcctgctacccgaggagcaaacgtagagcagtttctaatgatttatttaaaatatagaatcaaaagtaccagtttgcaattttgaaagatttatttcagcaatgcaacaacatcaggtggtgccgagtccaacacgtcttatgtcccatgatataaacaaaggccatccagaactgtggactggagttctaccttgtcccctaatgacattcagattttttttccattctctttatcttagaggagacagggggctaactcattttacttgtcctttgcttgttcttgccaagaacgtaaagcagcttgcaagtcttcaaacctaaatatcttagtaactcctacacgagtggcaatgccaaagagcagtgcaacaaagaggaagtaaatacgaccaaagagtattcttaaatacactactggctctaggttctgttttattatgcgcctttgaaccggaggggacccactgtctatgctcccactgtgtccctcttctttgcactttggagggctccaaccaaaatggcaatggcaattccgacgattgttacacactcctctgaaattgcatttttctggggtgcagtcataacccaaacgagataaacttccattgcaagctcctcgatcacagaacttaccccttgaacacggggtaccatgtctcaccaatccagcatctgctgtttctgtcccacgatgttcatcaagcccaaagcaggtaaccccagagataaccgattgatggaatgaaacatgttcttgcaaaaatggaagattggtgacattggtacactgcaaccttccacacagcttgtcctgatcagcacaagcattgaatgtgaggctttcttctgctctagtacaatgcccaaatcgaaaccgttgtttgttgatgtcatagcacttaatattagcattcttagcacttacaccaaagatttccatgcattgtatgttgcgatcagtgcagttacctttatagcagtaaccctcttctgagcatggtgtcccatcttgcagataagtgtcatctgggcaaatgaacttagagccactacagtactctggaagatcacatatgttctggataggtctgcagagtgtcccagaaggactgtaagtgcaatttgcacagcataattctttatcacaaatgctaccaggtgttaacctgcaatcatttccacagcagggatctgaataacatgccttttgggagccacagtcacactgctcattgttatctactttgaagtttccacaaaacttataagtcaatgatgtattataataaacatgacggtcatagaaaagacatggcatcagatcaggagtattaagtatgttgcttatctctgcaagggaacaattgctgaaagcatctgttaattgaggatttttgaacatgatgcaggtgttccttctctggcagatacagtacccctcatcatgttttaggcctaaactccttccaacacgattggttattataatagataaaaataaaggatttcgaccatgttgaccaagacaaattagggctgagggagaacatatactcctctcagctggattaacagcatcatctcctggcgaattcttgttaattatagctcctgcatcaggcctaaaatgagcataaaatactctctcatagaaagtatgagcctgccctcctggaactcgaaaatcttgtgaaaatggatcagcctcggtatacacagtcatgagaaagacatagtaccgcatatgaagattggtcagataggtgtccattaaactaatgactttaaacaaatactcaacagtagatgaaagtttgtcacctccagaagcactatatacagaatgggttgcttgaaagtggccttttatagcagctggatgtgtagcgtaattcttactagatagtctgggagctccatctgcatattccaatctggaggagggagaacctgtattatggctccagtgcttccatgcattcataggccctgtgtcatcagactcagatactatctgagaaacaaggtgttcaaagctctgtgaatcattgaggggtttgatttcataggtaaggttatccaactttatgacccctgacaggcccccataacaagtatccacagtgaccatggattgcaggatcccctccaggtagccaatatagtaacaatctacaggaaaaaaggggtactccatctgtaaggctccttggtcatcttgagttgtcagcaacaagtgtctgggccaaatgagtgtctttctccgcaggtggatgatatgtctctggccccgaaaacgcaagctatacgagagcagtctttgtgcttgaagtcctttggtatggtagatctccttccgaggaataaccacctccgatgagatgtaacgccaagtgggatggccttgagaacaccagactggaaccaggaggagcagccagagtgcaaatagcaagaggaggaccctggggaccacaggtctttccactagcctcatgccccaggtcagagataacatcctgggtggagctaactccctctgctgtggccactgcctggtctagaaaatactgacagaggactaaaaacctcctcaggctcccaacctaagtggttacccagacaactggagttaggtaacagtcactgggtgtggcaggaattgagtctgaatgtgttagctgaggttgaggttaaatattgtcaaaagggatgtctataaatgtgcctggacaagaaaagtcagaagcagcaaggagtgtctctgacaggctcaatcctttcttttctttttttgaagttcaaaatatcatttccacgtgaatgtatttggttcccagtgtgactctgggtctctttctaggagtcaatatttctttatatcttggctcatgtttttcacagttgttctaacttcttgttttgttttgtttgtttgtttgtttgaaagttagaagtaaatactgtctatattagccttttagctataaatgattgtttttatttcttctaatcatgttttgtttgagttttggttaaactatttacaaatgagttttttttttccttttgggtgttgctcgaaagtttggagctttctgttaatattgtgttgttgtttctccaatattattagacctgagaattctacctgggtacctgtgaactccagaatttttaaaaattccatctcttgggaacattatctctgaccccgtctgaggccgaagtggctgtccccctccaacctttagtatctttctttcctgactattgggatttcttcaagcaatcaggctgatgggttctcagcagtgagaccagtagactgtcggtatgaacgtcgaagagtctgccacacactccgggttcatcaacagtgctttcgcgtctcttacttttgtagaaggaaatgcagcctctgagttttctccaagaaatcattgatgaaagggtgaaaagatgggtatcacccggagttcatgacaagccctggctcagacacgtgagcaaggtctacagccccaaagataggctgccctgcaacatgtatttataagataggagaaaaaaatgggtagttggagggttgatcaacttacttcctctcaaacatatatatctcatctaagtgtgcaggggaaaactctgtagaactactgggatacctgctcacccccaggagcctcatgaataagtctctgcttctgccttgtagccatgagcattactgcacctgatacccctgcagcttcctagggaagagggaggaagtgacttggcccctgtctggttaaggtaagaggagataaatcccttctcattgattagggtgagaggggtcatgtgctctatcattggtgacccagttgggacatgggtttataccaaagtcatcactctgaggttctgtgtaccaccaggctgaactcccatatcctacatggacataggacaacaccaagcagaaggaggttttaggactaaactgaaggacagagatgcggtttctaaacaactagggagtgccagggccagcctctctaaccactataggacactgtggagtctggttacaaagagagattactcaaggtccttagcactgattacagagcatatctcagatgccttctgctgaccagatgtatctttgcataatctgcctatccagattcagaaaattgatgccacatagccaagtggactttcaggaacagacgatttaaaaacaggcagagagatgtgagagaaaggagaaggagagagagaagggagagggagagaagagagagggagacggagaaggaaagagggagaaggagaaggagagaaggggcatggacagagggagggacagaaggagagaggagatagagagggggataaggaagaagggagggagggagagagagagaaggctaagtctttccatacctgggtcccaatacctcttataacccaagcacatggtttcacatatcacaatgcggttgggatatagataactgtaaatacttgtgaaaataatggggctgagatctggggttttcatgatagtttcaaagtcaccgtactgactaaaaccttccactggcccatctccagcttcctaatctgagggtatcaaatttcccactaagtgtgtttagaaagatctccacctttttgcccttgtcttccagtgccccacctacgttctggtctcccacatctgatgtcttctcagtgattctggccctgcctgctccacagctacaaaccccttcctataatgagctctgtgctgagccatcatcctgaatcaatccaccttaagcagatgttttgcttatttttcctgtgtccatactacagaggaaaggtaggcatgtagaagctgaagcatctcacctcattccaagcaccctcagtctctaaatgtgcccccttgtttccagaagtgcaacctcaagcatcttttattcattcatcttagagggccacatgtgctgtagtgttataagatgaaatttaaagcattaattattcctaacaagccaattaaacaagccaaaaacattcatcagtcattcccatggaacctctgaagcatcttcctgctctaaccttgggttttccagggctgctctgggatcacaggagctgtcctgtctaccagccatataaaggcagacctatcagaattacaccagacttctcaccatagactataaaagccagaatatcctggacagatgttatacagaaactaagagaacacaaatgccagcccaggctactatacccagcaaaactctcaattaccatcgatgaagaaaccaagatattccattacaagtccaaatttacacaatatctttccataaatccagccctacaaaggatagcagatggaaaactccaacacaggtaggaaaactacaccctagaaagagcactaaagtaatcatctttcaacacactcaaaagaagataaccacacaaacataattccacctctaacaacaaaaataaagtaggcaacaatcactattccttaatatctcttttaacatcaatggactcaattctccaataaaaagacatagactaacagactgaatacataaacaggacacagcattttgctgcataaagcaaacacagcgttacttttttttttctaaatgacattttttattagatattgtctttattgacatttcaaatgttatcccctttcctggtttaccctctgaaatcccctatctcctccccctccccctgctcaccaatccacccactcccacttccaggccctggcaatcccctatatttgggcatagagccttcacaggaccaaggtactctccttgcattgatgaccaactagtccattctctgctacaaatgcagctagatctatgagtcccaccatgttttcttttgttggtggtttcatgccagggagctcttggagtactgattggttcatattgttgttctccctatggggttacaaaacccttcaacttcttgggtcctttctctggctgcctcattggggaccttgtgcgaagtccaatggatgactgtgagcatccacttctgtatttgccaggcactggcagagcctctcagaagacagctatatcaagatcctggcagcaagctcttgttggtatccacaaaagtgtctggtggttgtctatgggatggatccccaaaggggcagtctctggatggtcattccttcagtctctgttccacactttgtctctttaactccttccatgactattttattcctccctctaagaaggaccgaagtattcatactttggtcttccttcttgaaattcatgtgttttgtgaattgtatctttgatattccgaacttctgggctaatatccacttatcagtgagtgaatatcatgtgtgttcttatgtgattgagttacctcactcaggatgatatcctccagaaccatccatttgtctaagaatttaatgaattcattgtttttaatagctgaggagtactccattgtgtaaatgtaccacattttctgtacccattgttctcttgagggacatctgggttctttaaagcttctggacattaaatataaggctgctatggaaatagtggagaatgtgtccttattacatgttggagcatcttctgggtatatgcccaggagtgctattgctggatcctctgatagtactatgtccaattttctgaggaactgccaaactgatttacagagtggttgtaccagcttgcaattccaccagcaatggagaaatgttccccttcctccacatcctcaccaacatctgctgtcacctcaatttgttcttagtgattcagacaggtgtgaggtggaatatcagggttgtttggcatttccctgatgactagtgatattgaaaaaaattttaagtgtttctcagccattcagtattcttcagttgagaattcactgtttagctctgtactcaggtttttttaatagggttatttggttttctggagtctaacgtcttgaattctttctatatattggatattagccctctgtcatatttaggattggtaaagatctttcccaatatgttggctgcctttttgtgtcctttgccttacagaacctttttaattttatgaggtcccatttgctaattcttcattttacagcacaagccattggtgttctgttcaaaaatctttccccctgaaccctatcttcgaggatcttccccactttctcctctataagtttcagtgtctctattattgtgctgaggggtaccgaagttcctattccgaagttcctattctctagaaagtataggaacttccctagggtttaaacccgcggtggagctctgatgtgggaacgcttcagtgttcaggaaccatatgatttatttaaaatatagaatcaaaagtaccaatttgcagttttgaaagatttattccagtgtaagcattagcaatgcaccaacatcaggtgatttctgaatccaacacgtcttatgtcctcatgatattaaaaaaaaaaaaaggccatccagaactgtgaacttgagttctaccttgttccctactgacattcagattttcttttttgcattctctttatcttacaggagacaggaggggagggctaactcattttactttggcttgtcccttgctggtccttgcccagaacgtaaagtagcttgcaagtcttcaaatctaaaaatcttagtaactcctacacgagtggcaatgccaaagagcagtgcaacaaagaggaagtaaatacgaccaaagagtattcttaaatacaccactggctcttgtttttgttttattgtgtgcctttgaactggaggggacccactgtctatgctcccacttagtccctcttctttgcactctggaggcttccaaccaaaatgacaatggcaattccgatgattgttacacactcctctaaaactgcatttttctggggtgcagtcataacccaaatgagataaacttccactgcaagctccttgatcacagaacttacttttggagcagggggtaccatgtctcaccattccagcatctgttgtttctgtcccacgatgttcatcaagcccaaagcaggtaaacccagagataatcgattgatggaatgaaacatgttcttgcaaatatggaagattggtgacattggtacactgcaaccttccacacagcttgtcctgatcagcacaagcattgaatgtgaggctttcttctgctctagtacaatgcccaaatcgaaaccgttgtttgttgatgtcatagcacttaatattagcattcttagcacttacaccaaagatttccatgcattgtatgttgcgatcagtgcagttacctttatagcagtaaccatcttctgagcatggtgtcccatcttgcagataagtgtcatctgggcaaatgtatttagtcccattacagtactctggaagatcacatatgttctggataggtctgcagagtgtcccagaaggactgtaagtgcaatttgcacagcataattctttatcacaaatgctaccaggtgttaacctgcaatcatttccacagcagggatctgaataacatgccttttgggagccacagtcacactgctcatcgttatctactttgaagtttccacaaaacttataagtcaatgatgtattataataaacatgacggtcatagaaaagacatggcatcagaccaggagtattaagtatgttgcttatctctgcaagggaacaattgctgaaagcatctgttaattgaggatgtctgaacataatgcaggtgttccttctctggcagacacagtacccctcatcatattttaagcctaaactccttccaacacgattggttattataggagataaaaataaaggatttcgatcatatttaccaatacaaattagggctaaggaagaacatatactcctctcagctggattaacctggttatcttgtggcccatacttattaagtaaaactcctgcatcaggcttaaatttattataaaagactgacacatagtaattataagccgaccctcctggaactgcaaactcaagtcgaaatggatcagaattggtgtacacagtcatgagaaagacatagtaccgcatatgaagattggtcagataggtgtccattaaactaatgacttgaaacaaatacccaacagtagatgaaagtttgtcacctgcagcagaattatatacagaattggttgcttgaaagtggccttttatagcagctggatgtgtagcgtagttcttactagatattctgggagctccatctgcatattccaatctggaggagggagaacctgtattatggctccagtgcttccatgcattcataggccctgtgtcatcagactcagatactatctgagaaacaaggtgttcaaagctctgtgaatcattgaggggtttgatttcataggtaaggtcatctaacttcatgacccctgacaggcccccataacaagtatccacagtgaccatggattgtgggatcccctccaggtagccaatatagtaacaatctacaggaaaaaaggggtaatccatctgtaaggctccttggtcatcttgagttgtcagcaacaagtgtctgggccaaatgagtgtctttctccgcaggtggatgatatgtctctggccccgaaaatgcaagctatatgagagcagtctttgtgcttgaagtcctttggtatggtagatctccttccgaggaataaccacctccgatgagatgtaacgccaagtaggatggccttgagaacaccagactggaaccaggaggagcagccagagtgcaaatagcaagaggaggaccctggggaccacaggtctttccactagcctcatgccccaggtcagagataacatcctgggtggagctaaatccctctgctgtggccactgcctggtctagaaaatactgacagaggactaaaaacctcctcaggctcccaacctaagtggttacccagacaactggagttaggtaacagtcactgggtgtggcaggaattgagtctgaatgtgttagctgaggttgaggttaaatattgtcaaaagggatgtctataaatgtgcctggacaagaaaagtcagaagcagcaaggagtgtctctgacaggctcaatcctttcttttctttttttgaagttcaaaatatcatttccacgtgaatgtatttggttcccagtgtgactctgggtctctttctaggagtcaatatttctttatatcttggctcatgtttctcacagttgttctaatttcttgttttgttttgtttgtttgtttgaacgttagtagtaaatactgtctatattagccttttagctataaatgattgtttttatttcttctaatcatattttgtttgagttttggttaaactatttacaaatgagttttttttttttccttttgggtgttgctcgaaagtttggagctttctgttaatattgtgttgttatttttccaatattattagacctgagaattctatctgggtacctgtgaactctagaatttttaaaaattccatctcttgggaacattacctctgaccccgtctgaggccgaagtggctgtccccctccaacctttagtatctttctttcctgactattgggatttcttcaagcaatcaggctgatgggttctcagcagtgagaccagtagactgccggtatgaacgtcgaagagactgccacacactccaggttcatcaacagtgctttcgcgtctcttacttttgtagaaggaaaagcagcctctgagttatctccaagaaatcattaatgaaagagttaaaagatgggtatcacccggagttcatgacaagccctggctcagacacgtgagcaaggtctacagccccaaagataggctgccctgcaacatgtatttataagatagaagaaaaaaatgggtggttggagggttgatcaacttacttcctctcaaacatatatatctcatctaagtgtgcaggggaaaactctgtaggactactgggattgttattatcattattattattattattattattattattattattattattattaacttaaggcattttattagatattttcttcatttagttttcaaatgttatccccggaacctcctatactctctccctgccctgctccccaacccacccactcctacatcctggccctggcattcccctatactgtggcagatgatcttcgtaagaccaagagcctttcctcccattgatggcctactaggctatcctcttttacatatgcaactagagtcacagctctggggaggtattgcttagttcatattgtttttcctcctatagggttgcagatccctttagctccttgggtactttctctagctcctccattgggggccctgtgttccatccaatagatgactgtgagcatccacttctgtatttgccaggtattggcatggatcttactgcaccttctgaactctctaagcagctttcctggtcacctccaggagcctcatgaataagtctctgcttcccccttgtggctatgagcattactgcacctgatacaccctgcagcttcctagggaagagggaggaagtggcttggcccctgtctggttaaggtaagaggagataaatcccttctcatgaattagggtgagaagggtcatgtgctctatcattggtgaccaacttggggacatgggcttatacagtcatcactctgaggctctgtgtaccaccagactgaactcccatatcctacatgcacataggacaacaccaagtagaaggaggttttaggactaaactgaaggacagagatggggtttctaaacaactagggagtgccagggccagcctctctaaccactataggacactatggagtctggttacaaagagagattactcaaggtccttagcactgattacagagcatatctcagatgccttctgctgaccagatgtatctttgcataatctgcctatccagattcagaaaattgatgccacatagccaagtggactttcaggaacagacgatttaaaaacaggcagagagatgtgagagaaaggagaaggagagagagaagggagagggagagaagagagagggagacggagaaggaaagagggagaaggagaaggagagaaggggcatggacagagggagggacagaaggagagaggagatagagagggggataaggaagaaaggagggagggagagagagagaaggctaagtctttccatacctgggtcccaatacctcttataacccaagcacatggtttcagatatcacaatgcggttgggatatagataactgtaaatacttgtgaaaataatggggctgagatctggggttttcatgatagtttcaaagtcactgtactgactaaaaccttccactggcccatctccagcttgttaatctgagggtatcaaatttcccactaagtgtgtttagaaagatctccacctttttgccctagtcttccagtgccccacctacgttctggtctcccacatctgatgtcttctcagtgattctggccctgcctgctccacagctacaaaccccttcctataatgagctctgtgctgagccatcatcctgaatcaatccaccttaagcagatgttttgcttatttttcctgtgtccatactacagaggaagggtaggcatgtagaagctgaggcatctcatctcactctaagcaccctcagtctctaaatgtgcccctttgtttccagcagttcagcctcaagcatcttttattcactcgtcttagagggacacatgtgctgtagtgttataagatgaaatttaaagcattagttattcccaacaagccaattaaacaagccaaaaacattcatcagtcattcccatggaacctctgaagcatcttcctgctctaaccttgagtttcctagggctgctgtgggatcacaggagctgtcctgtttaccagcctatcctgtcccacgggattcagttattagtgggtgcgagggggaccgcaaacctggaagaaaatgggattggaagagaaaagagaaacgaagaccaagtagatcttttcctatcaaggtcttcgtttattaggctgaggtgcctggtgtaaagcatgcatcgcggggaataggaaggggtcgagggggaattttacaaagaacaaagaagcgggcatctgctgacatgagggccgaagtcaggctccaggcagcgggagctccaccgcggtggcgccatttcattacctctttctccgcacccgacatagataaagctta

SEQ ID NO: 4 - DNA, 251 bp, Artificial Sequence
  synthetic
ccagcttcattagtaatcgttcatctgtggtaaaaaggcaggatttgaagcgatggaagatgggagtacggggcgttggaagacaaagtgccacacagcgcagccttcgtctagacccccgggctaactataacggtcctaaggtagcgaggggatgacagattctctgttcagtgcactcagggtctgcctccacgagaatcaccatgccctttctcaagactgtgttctgtgcagtgccctgtcagtgg

SEQ ID NO: 5 - DNA, 245 bp, Artificial Sequence
  synthetic
aggggtcgagggggaattttacaaagaacaaagaagcgggcatctgctgacatgagggccgaagtcaggctccaggcagcgggagctccaccgcggtggcgccatttcattacctctttctccgcacccgacatagataaagcttatcccccaccaagcaaatccccctacctggggccgagcttcccgtatgtgggaaaatgaatccctgaggtcgattgctgcatgcaatgaaattcaactag

SEQ ID NO: 6 - DNA, 21 bp, Artificial Sequence
  synthetic
caggtacagctgcagcagtca

SEQ ID NO: 7 - DNA, 21 bp, Artificial Sequence
  synthetic
ggagatggcacaggtgagtga

SEQ ID NO: 8 - DNA, 17 bp, Artificial Sequence
  synthetic
tccaggactggtgaagc

SEQ ID NO: 9 - DNA, 24 bp, Artificial Sequence
  synthetic
tagtcccagtgatgagaaagagat

SEQ ID NO: 10 - DNA, 24 bp, Artificial Sequence
  synthetic
gagaacacagaagtggatgagatc

SEQ ID NO: 11 - DNA, 17 bp, Artificial Sequence
  synthetic
tgagtccagtccaggga

SEQ ID NO: 12 - DNA, 28 bp, Artificial Sequence
  synthetic
aaaaattgagtgtgaatggataagagtg

SEQ ID NO: 13 - DNA, 21 bp, Artificial Sequence
  synthetic
aaccctggtcagaaactgcca

SEQ ID NO: 14 - DNA, 19 bp, Artificial Sequence
  synthetic
agagaaacagtggatacgt

SEQ ID NO: 15 - DNA, 22 bp, Artificial Sequence
  synthetic
aactacgcacagaagttccagg

SEQ ID NO: 16 - DNA, 18 bp, Artificial Sequence
  synthetic
gctcgtggatttgtccgc

SEQ ID NO: 17 - DNA, 16 bp, Artificial Sequence
  synthetic
cagagtcacgattacc

SEQ ID NO: 18 - DNA, 19 bp, Artificial Sequence
  synthetic
tgagcagcaccctcacgtt

SEQ ID NO: 19 - DNA, 23 bp, Artificial Sequence
  synthetic
gtggcctcacaggtatagctgtt

SEQ ID NO: 20 - DNA, 18 bp, Artificial Sequence
  synthetic
accaaggacgagtatgaa

SEQ ID NO: 21 - DNA, 33 bp, Artificial Sequence
  synthetic
gctagtagtggggcctacaggccttttgatatc

SEQ ID NO: 22 - DNA, 48 bp, Artificial Sequence
  synthetic
gcaaaagcccaggggagtgggagctactacacctatgcttttgatatc

SEQ ID NO: 23 - DNA, 42 bp, Artificial Sequence
  synthetic
gcgagagagggtatagtgggaactactgaggactttgattac

SEQ ID NO: 24 - DNA, 33 bp, Artificial Sequence
  synthetic
gcgagagggacagtgggagccctctttgactac

SEQ ID NO: 25 - DNA, 36 bp, Artificial Sequence
  synthetic
gcgaaacctagtgggagctactcctggttcgacccc

SEQ ID NO: 26 - DNA, 45 bp, Artificial Sequence
  synthetic
gcgagaggaggagggtataactggaactcgaatgcttttgatatc

SEQ ID NO: 27 - DNA, 33 bp, Artificial Sequence
  synthetic
gcgagaggatataactggaactactttgactac

SEQ ID NO: 28 - DNA, 39 bp, Artificial Sequence
  synthetic
gcgaaagagtataactggaaccactggtactttgactac

SEQ ID NO: 29 - DNA, 33 bp, Artificial Sequence
  synthetic
gcgagagagataactggaaccccctttgactac

SEQ ID NO: 30 - DNA, 39 bp, Artificial Sequence
  synthetic
gcgaggggatataactggaacttttctttttttgactac

SEQ ID NO: 31 - DNA, 36 bp, Artificial Sequence
  synthetic
gcgagaggtaactggaactctctgggctttgactac

SEQ ID NO: 32 - DNA, 39 bp, Artificial Sequence
  synthetic
gcgaaaagggctactatggttcggggagctcttgactac

SEQ ID NO: 33 - DNA, 60 bp, Artificial Sequence
  synthetic
gcgagagatattactatggttcggggagttattataacgaaggtctacggtatggacgtc

SEQ ID NO: 34 - DNA, 27 bp, Artificial Sequence
  synthetic
gcgagagagtatagcagctttgactac

SEQ ID NO: 35 - DNA, 33 bp, Artificial Sequence
  synthetic
gcgagagagagtatagcagctcgttgtgactac

SEQ ID NO: 36 - DNA, 42 bp, Artificial Sequence
  synthetic
gcaagagaggataggagctcgcccctcgggtactttgactac

SEQ ID NO: 37 - DNA, 24 bp, Artificial Sequence
  synthetic
gcgagagatcttggggaaggctac

SEQ ID NO: 38 - DNA, 30 bp, Artificial Sequence
  synthetic
accacccataactggggagggtttgactac

SEQ ID NO: 39 - DNA, 18 bp, Artificial Sequence
  synthetic
gcgagagataggggaccg

SEQ ID NO: 40 - DNA, 30 bp, Artificial Sequence
  synthetic
caacagagttatagtacccctccggagacg

SEQ ID NO: 41 - DNA, 27 bp, Artificial Sequence
  synthetic
caacagcttaatagttaccctcggacg

SEQ ID NO: 42 - DNA, 26 bp, Artificial Sequence
  synthetic
caacagcttaatagttaccattcact

SEQ ID NO: 43 - DNA, 27 bp, Artificial Sequence
  synthetic
caacattttaatagttacccgctcact

SEQ ID NO: 44 - DNA, 27 bp, Artificial Sequence
  synthetic
cagcagtataataactggcctctcact

SEQ ID NO: 45 - DNA, 27 bp, Artificial Sequence
  synthetic
ctacagcataatagttacccgtggacg

SEQ ID NO: 46 - DNA, 27 bp, Artificial Sequence
  synthetic
ctacagcataatagttaccctcggacg

SEQ ID NO: 47 - DNA, 27 bp, Artificial Sequence
  synthetic
cagcagtatggtagctcacctcggacg

SEQ ID NO: 48 - DNA, 27 bp, Artificial Sequence
  synthetic
atgcaaggtacacactggccgtggacg

SEQ ID NO: 49 - DNA, 27 bp, Artificial Sequence
  synthetic
atgcaaggttcacactggccgtacact

SEQ ID NO: 50 - DNA, 27 bp, Artificial Sequence
  synthetic
atgcaaggtacacactggccgctcact

SEQ ID NO: 51 - DNA, 27 bp, Artificial Sequence
  synthetic
caacagtatgataatctccctcccact

SEQ ID NO: 52 - DNA, 27 bp, Artificial Sequence
  synthetic
caacagtatgataatctcccattcact

SEQ ID NO: 53 - DNA, 27 bp, Artificial Sequence
  synthetic
caacagtatgataatctccccgtcact

SEQ ID NO: 54 - DNA, 27 bp, Artificial Sequence
  synthetic
caacagtatgataatctcccgatcacc

SEQ ID NO: 55 - DNA, 24 bp, Artificial Sequence
  synthetic
caacggatttacaatgccgacacc

SEQ ID NO: 56 - DNA, 30 bp, Artificial Sequence
  synthetic
caacagagttacagtacccccatgtacact

SEQ ID NO: 57 - DNA, 27 bp, Artificial Sequence
  synthetic
caacagagttacagtacccctctcact

SEQ ID NO: 58 - DNA, 27 bp, Artificial Sequence
  synthetic
caacagagttacagtactcctcccact

SEQ ID NO: 59 - DNA, 3155 bp, Artificial Sequence
  Synthetic
ggcgcgccgtagctttgaattttaaacatctatttgacaagaaatgcatagttccttctctttaaaataatgtaatgtttctttcaagaataagcttggtttgatgcctctctccccaacatgatagaagtgtagcataaatctatgaaaaattccatttccctgtgcctacaacaactacctgggattgaaaacttcttcccttgctctagtcctttcttctacacctacttccacatcatctgtgactcaaaacaatacttgtcaggaaagatcccggaaagagcaaaaaagacttccttagaggtgtcagagattcctatgccactatctgtcatctctagaaggggttgtgagtatgaggaagagcagagcttgtaaattttctacttgctttgacttccactgtatttcctaacaacaacaaccacagcaacacccataacatcacaggacaaacttctagtacttccaaggctttagtctcagtaaatcttctctacctccatcacagcagctagaaggtttgatactcatacaaatagtactgtagctttctgttcataattggaaaaatagacaagacccaatgtaatacaggctttccttcagccagttagcgttcagtttttggatcaccattgcacacatatacccagcatatgtctaatatatatgtagaaatccgtgaagcaagagttataatagcttgtgttttctattgtattgtattttcctcttatatcatcttcttcttcgttcattaaaaaaaaaccgttcaagtaggtctaaattaattattggatcataagtagataaaatattttatttcataacacattgacccgatgaatatgtttctttgccagacatagtcctcatttccaaggtaacaagcctgaaaaaattatactggagcaagtcaacaggtaatgatggtagcttttccttattgtcctggggcaagaataagacaaaagataacagggtagaataaagattgtgtaagaaagaaggacagcaacaggacatgggaaccttttatagagtaacattttgataatggatgatgagaattaatgagttagacagggatgggtgggaatgattgaaggtgtgagtactttagcacagattaagaccaaatcattaggatttaaagagttgtgtagagttagtgaaggaaaagccttagaattaaatttggctgcggataaaacattcttggattagactgaagactcttttctgtgctaagtaagtatatttatgataatgatgatgactgtagtgctgaatatttaataaataaaaacaaaattaattgccgcatacataatgtcctgaatactattgtaaatgttttatcttatttcctttaaactgtctacagcactataaggtaggtaccagtattgtcacagttacacagatatggaaaccgagacacagggaagttaagttacttgatcaatttcaagcaatcggcaagccatggagcatctatgtcagggctgccaggacatgtgactgtaaacagaagtttttcactttttaactcaaagagggtatgtggctgggttaatggaaagcttcaggaccctcagaaaacattactaacaagcaaatgaaaggtgtatctggaagattaagttttaacagactcttcatttccatcgatccaataatgcacttagggagatgactgggcatattgaggataggaagagagaagtgaaaacacagctttttatattgttcttaacaggcttgtgccaaacatcttctgggtggatttaggtgattgaggagaagaaagacacaggagcgaaattctctgagcacaagggaggagttctacactcagactgagccaacagacttttctggcctgacaaccagggcggcgcaggatgctcagtgcagagaggaagaagcaggtggtctttgcagctgaaagctcagctgatttgcatatggagtcattatacaacatcccagaattctttaagggcagctgccaggaagctaagaagcatcctctcttctagctctcagagatggagacagacacactcctgctatgggtgctgctgctctgggttccaggtgagggtacagataagtgttatgagcaacctctgtggccattatgatgctccatgcctctctgttcttgatcactataattagggcatttgtcactggttttaagtttccccagtcccctgaattttccattttctcagagtgatgtccaaaattattcttaaaaatttaaatgaaaaggtcctctgctgtgaaggcttttaaagatatataaaaataatctttgtgtttatcattccaggtgccagatgtgacatccagatgacccagtctccatcctccctgtctgcatctgtaggagacagagtcaccatcacttgccgggcaagtcagagcattagcagctatttaaattggtatcagcagaaaccagggaaagcccctaagctcctgatctatgctgcatccagtttgcaaagtggggtcccatcaaggttcagtggcagtggatctgggacagatttcactctcaccatcagcagtctgcaacctgaagattttgcaacttactactgtcaacagagttacagtacccctccgatcaccttcggccaagggacacgactggagattaaacgtaagtaatttttcactattgtcttctgaaatttgggtctgatggccagtattgacttttagaggcttaaataggagtttggtaaagattggtaaatgagggcatttaagatttgccatgggttgcaaaagttaaactcagcttcaaaaatggatttggagaaaaaaagattaaattgctctaaactgaatgacacaaagtaaaaaaaaaaagtgtaactaaaaaggaacccttgtatttctaaggagcaaaagtaaatttatttttgttcactcttgccaaatattgtattggttgttgctgattatgcatgatacagaaaagtggaaaaatacattttttagtctttctcccttttgtttgataaattattttgtcagacaacaataaaaatcaatagcacgccctaagatctagatgcatgctcgagtgccatttcattacctctttctccgcacccgacatagat

SEQ ID NO: 60 - DNA, 28 bp, Artificial Sequence
  Synthetic
aggtgagggtacagataagtgttatgag

SEQ ID NO: 61 - DNA, 27 bp, Artificial Sequence
  Synthetic
tgacaaatgccctaattatagtgatca

SEQ ID NO: 62 - DNA, 21 bp, Artificial Sequence
  Synthetic
gggcaagtcagagcattagca

SEQ ID NO: 63 - DNA, 21 bp, Artificial Sequence
  Synthetic
tgcaaactggatgcagcatag

SEQ ID NO: 64 - DNA, 19 bp, Artificial Sequence
  Synthetic
ggtggagaggctattcggc

SEQ ID NO: 65 - DNA, 17 bp, Artificial Sequence
  Synthetic
gaacacggcggcatcag

SEQ ID NO: 66 - DNA, 23 bp, Artificial Sequence
  Synthetic
tgggcacaacagacaatcggctg

SEQ ID NO: 67 - DNA, 29 bp, Artificial Sequence
  Synthetic
ccattatgatgctccatgcctctctgttc

SEQ ID NO: 68 - DNA, 26 bp, Artificial Sequence
  Synthetic
atcagcagaaaccagggaaagcccct

SEQ ID NO: 69 - DNA, 3166 bp, Artificial Sequence
  Synthetic
ggcgcgccgtagctttgaattttaaacatctatttgacaagaaatgcatagttccttctctttaaaataatgtaatgtttctttcaagaataagcttggtttgatgcctctctccccaacatgatagaagtgtagcataaatctatgaaaaattccatttccctgtgcctacaacaactacctgggattgaaaacttcttcccttgctctagtcctttcttctacacctacttccacatcatctgtgactcaaaacaatacttgtcaggaaagatcccggaaagagcaaaaaagacttccttagaggtgtcagagattcctatgccactatctgtcatctctagaaggggttgtgagtatgaggaagagcagagcttgtaaattttctacttgctttgacttccactgtatttcctaacaacaacaaccacagcaacacccataacatcacaggacaaacttctagtacttccaaggctttagtctcagtaaatcttctctacctccatcacagcagctagaaggtttgatactcatacaaatagtactgtagctttctgttcataattggaaaaatagacaagacccaatgtaatacaggctttccttcagccagttagcgttcagtttttggatcaccattgcacacatatacccagcatatgtctaatatatatgtagaaatccgtgaagcaagagttataatagcttgtgttttctattgtattgtattttcctcttatatcatcttcttcttcgttcattaaaaaaaaaccgttcaagtaggtctaaattaattattggatcataagtagataaaatattttatttcataacacattgacccgatgaatatgtttctttgccagacatagtcctcatttccaaggtaacaagcctgaaaaaattatactggagcaagtcaacaggtaatgatggtagcttttccttattgtcctggggcaagaataagacaaaagataacagggtagaataaagattgtgtaagaaagaaggacagcaacaggacatgggaaccttttatagagtaacattttgataatggatgatgagaattaatgagttagacagggatgggtgggaatgattgaaggtgtgagtactttagcacagattaagaccaaatcattaggatttaaagagttgtgtagagttagtgaaggaaaagccttagaattaaatttggctgcggataaaacattcttggattagactgaagactcttttctgtgctaagtaagtatatttatgataatgatgatgactgtagtgctgaatatttaataaataaaaacaaaattaattgccgcatacataatgtcctgaatactattgtaaatgttttatcttatttcctttaaactgtctacagcactataaggtaggtaccagtattgtcacagttacacagatatggaaaccgagacacagggaagttaagttacttgatcaatttcaagcaatcggcaagccatggagcatctatgtcagggctgccaggacatgtgactgtaaacagaagtttttcactttttaactcaaagagggtatgtggctgggttaatggaaagcttcaggaccctcagaaaacattactaacaagcaaatgaaaggtgtatctggaagattaagttttaacagactcttcatttccatcgatccaataatgcacttagggagatgactgggcatattgaggataggaagagagaagtgaaaacacagctttttatattgttcttaacaggcttgtgccaaacatcttctgggtggatttaggtgattgaggagaagaaagacacaggagcgaaattctctgagcacaagggaggagttctacactcagactgagccaacagacttttctggcctgacaaccagggcggcgcaggatgctcagtgcagagaggaagaagcaggtggtctttgcagctgaaagctcagctgatttgcatatggagtcattatacaacatcccagaattctttaagggcagctgccaggaagctaagaagcatcctctcttctagctctcagagatggagacagacacactcctgctatgggtgctgctgctctgggttccaggtgagggtacagataagtgttatgagcaacctctgtggccattatgatgctccatgcctctctgttcttgatcactataattagggcatttgtcactggttttaagtttccccagtcccctgaattttccattttctcagagtgatgtccaaaattattcttaaaaatttaaatgaaaaggtcctctgctgtgaaggcttttaaagatatataaaaataatctttgtgtttatcattccaggtgccagatgtataccaccggagaaattgtgttgacgcagtctccaggcaccctgtctttgtctccaggggaaagagccaccctctcctgcagggccagtcagagtgttagcagcagctacttagcctggtaccagcagaaacctggccaggctcccaggctcctcatctatggtgcatccagcagggccactggcatcccagacaggttcagtggcagtgggtctgggacagacttcactctcaccatcagcagactggagcctgaagattttgcagtgtattactgtcagcagtatggtagctcaccttggacgttcggccaagggaccaaggtggaaatcaaacgtaagtaatttttcactattgtcttctgaaatttgggtctgatggccagtattgacttttagaggcttaaataggagtttggtaaagattggtaaatgagggcatttaagatttgccatgggttgcaaaagttaaactcagcttcaaaaatggatttggagaaaaaaagattaaattgctctaaactgaatgacacaaagtaaaaaaaaaaagtgtaactaaaaaggaacccttgtatttctaaggagcaaaagtaaatttatttttgttcactcttgccaaatattgtattggttgttgctgattatgcatgatacagaaaagtggaaaaatacattttttagtctttctcccttttgtttgataaattattttgtcagacaacaataaaaatcaatagcacgccctaagatctagatgcatgctcgagtgccatttcattacctctttctccgcacccgacatagat

SEQ ID NO: 70 - DNA, 19 bp, Artificial Sequence
  Synthetic
tccaggcaccctgtctttg

SEQ ID NO: 71 - DNA, 26 bp, Artificial Sequence
  Synthetic
aagtagctgctgctaacactctgact

SEQ ID NO: 72 - DNA, 24 bp, Artificial Sequence
  Synthetic
aaagagccaccctctcctgcaggg

SEQ ID NO: 73 - DNA, 3187 bp, Artificial Sequence
  Synthetic
ggcgcgccgtagctttgaattttaaacatctatttgacaagaaatgcatagttccttctctttaaaataatgtaatgtttctttcaagaataagcttggtttgatgcctctctccccaacatgatagaagtgtagcataaatctatgaaaaattccatttccctgtgcctacaacaactacctgggattgaaaacttcttcccttgctctagtcctttcttctacacctacttccacatcatctgtgactcaaaacaatacttgtcaggaaagatcccggaaagagcaaaaaagacttccttagaggtgtcagagattcctatgccactatctgtcatctctagaaggggttgtgagtatgaggaagagcagagcttgtaaattttctacttgctttgacttccactgtatttcctaacaacaacaaccacagcaacacccataacatcacaggacaaacttctagtacttccaaggctttagtctcagtaaatcttctctacctccatcacagcagctagaaggtttgatactcatacaaatagtactgtagctttctgttcataattggaaaaatagacaagacccaatgtaatacaggctttccttcagccagttagcgttcagtttttggatcaccattgcacacatatacccagcatatgtctaatatatatgtagaaatccgtgaagcaagagttataatagcttgtgttttctattgtattgtattttcctcttatatcatcttcttcttcgttcattaaaaaaaaaccgttcaagtaggtctaaattaattattggatcataagtagataaaatattttatttcataacacattgacccgatgaatatgtttctttgccagacatagtcctcatttccaaggtaacaagcctgaaaaaattatactggagcaagtcaacaggtaatgatggtagcttttccttattgtcctggggcaagaataagacaaaagataacagggtagaataaagattgtgtaagaaagaaggacagcaacaggacatgggaaccttttatagagtaacattttgataatggatgatgagaattaatgagttagacagggatgggtgggaatgattgaaggtgtgagtactttagcacagattaagaccaaatcattaggatttaaagagttgtgtagagttagtgaaggaaaagccttagaattaaatttggctgcggataaaacattcttggattagactgaagactcttttctgtgctaagtaagtatatttatgataatgatgatgactgtagtgctgaatatttaataaataaaaacaaaattaattgccgcatacataatgtcctgaatactattgtaaatgttttatcttatttcctttaaactgtctacagcactataaggtaggtaccagtattgtcacagttacacagatatggaaaccgagacacagggaagttaagttacttgatcaatttcaagcaatcggcaagccatggagcatctatgtcagggctgccaggacatgtgactgtaaacagaagtttttcactttttaactcaaagagggtatgtggctgggttaatggaaagcttcaggaccctcagaaaacattactaacaagcaaatgaaaggtgtatctggaagattaagttttaacagactcttcatttccatcgatccaataatgcacttagggagatgactgggcatattgaggataggaagagagaagtgaaaacacagctttttatattgttcttaacaggcttgtgccaaacatcttctgggtggatttaggtgattgaggagaagaaagacacaggagcgaaattctctgagcacaagggaggagttctacactcagactgagccaacagacttttctggcctgacaaccagggcggcgcaggatgctcagtgcagagaggaagaagcaggtggtctttgcagctgaaagctcagctgatttgcatatggagtcattatacaacatcccagaattctttaagggcagctgccaggaagctaagaagcatcctctcttctagctctcagagatggagacagacacactcctgctatgggtgctgctgctctgggttccaggtgagggtacagataagtgttatgagcaacctctgtggccattatgatgctccatgcctctctgttcttgatcactataattagggcatttgtcactggttttaagtttccccagtcccctgaattttccattttctcagagtgatgtccaaaattattcttaaaaatttaaatgaaaaggtcctctgctgtgaaggcttttaaagatatataaaaataatctttgtgtttatcattccaggtgccagatgtgttgtggtcctcagccggtgctgcatcagccgccggccatgtcctcggcccttggaaccacaatccgcctcacctgcaccctgaggaacgaccatgacatcggtgtgtacagcgtctactggtaccagcagaggccgggccaccctcccaggttcctgctgagatatttctcacaatcagacaagagccagggcccccaggtcccccctcgcttctctggatccaaagatgtggccaggaacagggggtatttgagcatctctgagctgcagcctgaggacgaggctatgtattactgtgctatgcataactcagtgacgcatgtgtttggcagcgggacccagctcaccgttttaagtaagtaatttttcactattgtcttctgaaatttgggtctgatggccagtattgacttttagaggcttaaataggagtttggtaaagattggtaaatgagggcatttaagatttgccatgggttgcaaaagttaaactcagcttcaaaaatggatttggagaaaaaaagattaaattgctctaaactgaatgacacaaagtaaaaaaaaaaagtgtaactaaaaaggaacccttgtatttctaaggagcaaaagtaaatttatttttgttcactcttgccaaatattgtattggttgttgctgattatgcatgatacagaaaagtggaaaaatacattttttagtctttctcccttttgtttgataaattattttgtcagacaacaataaaaatcaatagcacgccctaagatctagatgcatgctcgagtgccatttcattacctctttctccgcacccgacatagat

SEQ ID NO: 74 - DNA, 17 bp, Artificial Sequence
  Synthetic
tgtcctcggcccttgga

SEQ ID NO: 75 - DNA, 20 bp, Artificial Sequence
  Synthetic
ccgatgtcatggtcgttcct

SEQ ID NO: 76 - DNA, 23 bp, Artificial Sequence
  Synthetic
acaatccgcctcacctgcaccct

SEQ ID NO: 77 - DNA, 23 bp, Artificial Sequence
  synthetic
agcagtctgcaacctgaagattt

SEQ ID NO: 78 - DNA, 24 bp, Artificial Sequence
  synthetic
gtttaatctccagtcgtgtccctt

SEQ ID NO: 79 - DNA, 15 bp, Artificial Sequence
  synthetic
cctccgatcaccttc

SEQ ID NO: 80 - DNA, 20 bp, Artificial Sequence
  synthetic
aaaccagggaaagcccctaa

SEQ ID NO: 81 - DNA, 18 bp, Artificial Sequence
  synthetic
atgggaccccactttgca

SEQ ID NO: 82 - DNA, 19 bp, Artificial Sequence
  synthetic
ctcctgatctatgctgcat

SEQ ID NO: 83 - DNA, 21 bp, Artificial Sequence
  synthetic
cagcagactggagcctgaaga

SEQ ID NO: 84 - DNA, 21 bp, Artificial Sequence
  synthetic
tgatttccaccttggtccctt

SEQ ID NO: 85 - DNA, 18 bp, Artificial Sequence
  synthetic
tagctcaccttggacgtt

SEQ ID NO: 86 - DNA, 22 bp, Artificial Sequence
  synthetic
ctcctcatctatggtgcatcca

SEQ ID NO: 87 - DNA, 20 bp, Artificial Sequence
  synthetic
gacccactgccactgaacct

SEQ ID NO: 88 - DNA, 13 bp, Artificial Sequence
  synthetic
ccactggcatccc

SEQ ID NO: 89 - DNA, 19 bp, Artificial Sequence
  synthetic
tgagcagcaccctcacgtt

SEQ ID NO: 90 - DNA, 23 bp, Artificial Sequence
  synthetic
gtggcctcacaggtatagctgtt

SEQ ID NO: 91 - DNA, 18 bp, Artificial Sequence
  synthetic
accaaggacgagtatgaa